European Patent Application EP 4 516 930 A2, published March 5, 2025. Title: TBRFV resistant tomato plants. Applicant: Rijk Zwaan Zaadteelt en Zaadhandel B.V. Application EP. The sequence listing filed with the application follows.

SEQUENCE LISTING (53 sequences)

SEQ ID NO: 1 - DNA, 201 bp, Solanum lycopersicum
  source 1..201: mol_type = genomic DNA
tttatgggacgttgagcatctcatgaacttacggagatttctagttgagttgtgtgatcaagtggtagatttaacgttgtgtactatctctaaaagcttggtcttaccaagaggaatttatcgtcttcctacacttgaagtcgagaatttggaactgtcttatagtgatattacaaccgcgacatattcattttactatga

SEQ ID NO: 2 - DNA, 201 bp, Solanum lycopersicum
  source 1..201: mol_type = genomic DNA
acacattaataagtttcaagtaccgataaaggcaaatttttatcatgggttagcaaagcaagatgagtaaggtatctgtagaattagatatactcaaccatgtctaaaaggtgtgtcactttcagatgcctacatttaccgaaaaaagataatcttgcttttatgggctttaaccaaatacacaagaatgggatgcaacag

SEQ ID NO: 3 - DNA, 201 bp, Solanum lycopersicum
  source 1..201: mol_type = genomic DNA
agaaacaacccctctacctaacacaaggtatgtgtaaggtctaagtagactctactatactagatatgttattgttgttgagaaatgtaatatgagggtcggaaacatccactctacctaacacaaggtatgtgtaaggtctacatagactattatactgaatatgttattgttgttgagaaatgtaatctgagggtcgga

SEQ ID NO: 4 - DNA, 201 bp, Solanum lycopersicum
  source 1..201: mol_type = genomic DNA
gagagagcgaatctgcaaagctgatttccgatgctactgcggctgctggaatgggtttgattgagctgaggaggattgaagcttctagagaagttgctgggactttggctaagactcctaatgttgcttacttgcctaagcaagggaatatgcttcttggactcggccgttgagtaggtaatcaattgagcaaaatgctag

SEQ ID NO: 5 - DNA, 201 bp, Solanum lycopersicum
  source 1..201: mol_type = genomic DNA
ttgtagttaactaattaaatttagaatmtycatcctacaacgcaagttaaaaacactcgtaaatccggacacatgttgtaggattaggggtagatgtttttgaggctattaatagtgtagagataaaagttttggagtgttttcaatacatctgtctygttagaaaaaggtcgaggcccacgttaaccggccattgtcacc

SEQ ID NO: 6 - DNA, 201 bp, Solanum lycopersicum
  source 1..201: mol_type = genomic DNA
gtttcattgtgttaagaattgtgcctgggaaaatgggtctctgatggaatggcaaaagaaagtttatgtgttactgaagcttttcggttattgaagaagaggaagaaaaaaactatatggggagttcacagcagtccggtagctttggggaccctcaacaaatctcctctgataatgttaatggtctttgcttggctattt

SEQ ID NO: 7 - DNA, 201 bp, Solanum lycopersicum
  source 1..201: mol_type = genomic DNA
tgagaagaaaagaagcagagttcaatgtaatgtcactacaactttctttattytgatctgaaagattgtcagctccacaaacagtaccagacacagacacgactgccacattgattaggaaggacacaaayaacgcgaaaccgctctctatcaagaagaatttacatgcatcctacaaaatycaacattaattaatttttc

SEQ ID NO: 8 - DNA, 201 bp, Solanum lycopersicum
  source 1..201: mol_type = genomic DNA
agctactatcarttttccaagaactttgcttctattgcaactcatttgactagtctgactcagaatgaagtgcctttagttgtagtccgaccagtgaaaaaagagctttcaaaagcgcaagacatttttgactatgatccmaacattaggggtggaaggtaatgactacattgtatrttgtgatgcttcacatttgggttt

SEQ ID NO: 9 - DNA, 201 bp, Solanum lycopersicum
  source 1..201: mol_type = genomic DNA
cactcgtgacatgccttcacttcatccccgttacccctcaacttataaaccccatattctatctatcaagacttatacccgcttcagtaccacatctttctgggtcaacattacaacatgtcaccacccccatcctcaatgacaatacacatgaccatatttctaaaacacaacaacaccgagacttttagtctccaccta

SEQ ID NO: 10 - DNA, 201 bp, Solanum lycopersicum
  source 1..201: mol_type = genomic DNA
attggtggtaatagagattctgtgactggtggtggtggtgattctgtgaytggtggaggaggtgattytgtgactggtggtggtggagatgtaggctaatttgattttggggaagatggagaagatgtagacggtttgtttgtggttgattttcttccccctgagcaggtactgtatcaatgamagggttctcttccccct

SEQ ID NO: 11 - DNA, 201 bp, Solanum lycopersicum
  source 1..201: mol_type = genomic DNA
ttaagagtttcaatatcctttgtggtatcgtcaagaaaatcttgcagagcagaaagatttttttggagagattcgacatgttgttgtgtacaacttcgacgaacgaaagattggttaggtttgaagagttgttctaatgtatacataagtgaagaaagagcagcataagccatttctcttaacaacaattattgctaaaga

SEQ ID NO: 12 - DNA, 201 bp, Solanum lycopersicum
  source 1..201: mol_type = genomic DNA
catcagattcctgcaaaatataattacacctcacttaagaagtacttgcctttaggtatgaagccacctgcaatatatttcagaaaaaacagtgaaaagtgacgagtcagtaaaaaaaatgaaacaagagtgtaaccaataaaattaaaaaaattctccttctcacccatgcgaaaagtgctgaaaaaccaacaccaactc

SEQ ID NO: 13 - DNA, 201 bp, Solanum lycopersicum
  source 1..201: mol_type = genomic DNA
agtccttatctattattatatggtgaacaagtcaataaaaatactcgtaattgaaatagttatcgataattgttcacttccctcttatggaattcgagtttacaattatgatgtgttgttgaatagtgtaagaattgatgcatcatcacttaaatatattctgttagaaatattattgaattcattgtacaatccatttgt

SEQ ID NO: 14 - DNA, 201 bp, Solanum lycopersicum
  source 1..201: mol_type = genomic DNA
ctcaatcgaaggtactttggaagtatcatccctgagatgtgccaagaaagctacacaacccttactcatcatcctgttagcacgaagaaaagagataatacgaactggagtggaaatttagtcaccctcccacactagcggatctgtcccaggcttggccaatattacagttttagcattacaatctaagattgcaaaatt

SEQ ID NO: 15 - DNA, 201 bp, Solanum lycopersicum
  source 1..201: mol_type = genomic DNA
tcaaatcatcaagaaacgtccatgacgtcaggaaactagttcaagaggtgttgatgtgcgttagcctatttgactaggttttaggagtcagaatttgatggaattcggtagtaaggtgtctaatacgtattcgagttgttttatagtcaaaaattctgggtacgactctccaaggaccaaccaaagggcccttgaggagga

SEQ ID NO: 16 - DNA, 201 bp, Solanum lycopersicum
  source 1..201: mol_type = genomic DNA
aattggcctttcctctttctagttgaaaaaaaaaacaaaacaaagaggtatatgcaccaattaacatcaattgtgaattcaccagtgacgatatctacttcaaaagatgtttgtcttctactgaatacaggatatgaattaaattttctagctccaagacaccaatttagcataactatakttataatactacaaaaaaaa

SEQ ID NO: 17 - DNA, 201 bp, Solanum lycopersicum
  source 1..201: mol_type = genomic DNA
aacaaacaatacgaaactctatgcctaaaaatacacatatcaacgaaactgacataacatatctcccattgattttaaaattgttgaaaatgcttacaattgttaattccactagatttgagagtagacaaacaattaatgaaactcaattcctaaaatacacatgaaaattaccataactatataaataaggtgattttt

SEQ ID NO: 18 - DNA, 201 bp, Solanum lycopersicum
  source 1..201: mol_type = genomic DNA
gcattaaaatccattgcattactaatgcatagaactccatggtattagtaatatgctaatgcatgcattagaatccattgcactactaatgcatagaacttcatggtattaataatactcttcaatacacaataaattgtattactaatacaagcattagttatgcatacgttagaaaagtgtactaaacaaggtactagt

SEQ ID NO: 19 - DNA, 201 bp, Solanum lycopersicum
  source 1..201: mol_type = genomic DNA
gcatgcatttagaagagaaatgctgttttataaacttcaactaaaataacctgcaatttctttaaacattgaagaaaggccatgagcaacattgctagggatgggttgggcaccctcatcaccaaggaccaatttagcatctgcattcatcaccgcaacatcaaacatgggacgtaatcccacgtagtgttgcatggcact

SEQ ID NO: 20 - DNA, 101 bp, Solanum lycopersicum
  source 1..101: mol_type = genomic DNA
aaatttcctcttttctacctcaaattcgtacagcaagagcatgcttggcatgagaccaaacacacgcggagattccggaggtaaccatggtatggtcatgt

SEQ ID NO: 21 - DNA, 201 bp, Solanum lycopersicum
  source 1..201: mol_type = genomic DNA
cacatattaatgaaaggaatatcccaattcaaattgatgtcaccataggaccatcaactagtggcatagctaatgagtcaaaagcacgcctaaagcgtggcaggccatttggatcaaaaccctagaaaatgaaaatcaaaagatcaaaatgacactatgaaaaaacctcacatagaaagtcaagacgtgagtaattctgat

SEQ ID NO: 22 - DNA, 201 bp, Solanum lycopersicum
  source 1..201: mol_type = genomic DNA
tcaatcaataggagcgacgggcggtgtgtacaaagggtagggacgtagtcaatgcgagctgatgactcgtgcttactaggaattccttgttgaaaaccaacaaatgcaatgatatatccctatcacgatgaaatttcaaagattacccgggcctattggccaaggctataaactcgttgaataatcagtgtagcgcgcgtg

SEQ ID NO: 23 - DNA, 201 bp, Solanum lycopersicum
  source 1..201: mol_type = genomic DNA
ttcaataagcttaatacttaatggatctaagaatatatattattcatttgatcaatttgagataaactataaaccatacaataataatctatacataaataaagagtctataacaatctatacatgaattcattaatatcaaagcatgatcacacaacccatatttaagtcaaattgagagatttgagaaggtcaagggtt

SEQ ID NO: 24 - DNA, 201 bp, Solanum lycopersicum
  source 1..201: mol_type = genomic DNA
ggaggtgtctggccctgatcagataacccgctaagataagccagaacctgattgatcatctctggggtaggttggggtggcatttcctcattctacactttttcattctcctcatcctccccttctcttactacttcctcagttggtggaggagtcaccgccctagtaccagatgggccaggcgttcgtcctcttcctcta

SEQ ID NO: 25 - DNA, 201 bp, Solanum lycopersicum
  source 1..201: mol_type = genomic DNA
ggaccttccacataagtttcaacaaaaacgaacacgtaaaacatgtaaaggtacaccaagacacacatgcatgtctcaagtctaaccttcaaacgtcatcagacattcttggacatttgacctccaaatgatttcaaattaatcatacattcttaaaacacttaattaacaggtgaacaagattattacacacatgtgagg

SEQ ID NO: 26 - DNA, 201 bp, Solanum lycopersicum
  source 1..201: mol_type = genomic DNA
gttgaaggttccacataaaggaccttattagaaacattcaaggtctcatgtcattcgtacatacaagactaagagactttagcatcctaattcaatacatatgatattcatattcatccatgtatcaagtaagggacacaagtctaccacacaagatacacaaatacttcactttaccccatataacatataattctagaa

SEQ ID NO: 27 - DNA, 201 bp, Solanum lycopersicum
  source 1..201: mol_type = genomic DNA
aaccaacattayacaattcatatcaagataacaacctrgggttaagtgttaaaggtcattttctacaaactagactgatttatcaacaaataacataattaagttaaagtacatgttaaactattcatgacatccataataaatcataaataaagtaattcacaagcccaatttcaagatttgaaaagactcacttgaatt

SEQ ID NO: 28 - DNA, 201 bp, Solanum lycopersicum
  source 1..201: mol_type = genomic DNA
cgctaaaggaaccgaataaaatgggagatcttcggagagaatggattttgttgaagttggggaagtgtggaatcttgtgatggaatgagagtgaatgggttaggtagtggggggaaaaaagaggaaatagggagggaaacggttaagggggttatgtaaagaggtgggtaactgaagagtttaaaaacttttcatatgtag

SEQ ID NO: 29 - DNA, 201 bp, Solanum lycopersicum
  source 1..201: mol_type = genomic DNA
aactctcatactcgttcattcaatgtcctgatttttgttggcctgtatcgtatcatgatgcatacgcaggtaacgaggatcgacatccaatgcatcattggttcagttgagcactccagagtcggttggtgcgcctctttgctttttggaggatccattttatttctttctagtttagtttattaggatctgtcccaacac

SEQ ID NO: 30 - DNA, 201 bp, Solanum lycopersicum
  source 1..201: mol_type = genomic DNA
gatttaatgaacaagatattcaaacaatatttggacttgtttgtcattgtctttatttataatatcccgatttattctcaaagtgagaaagagcatccgaaccatatgagagtttctatgcaaactctcaaagatcgacaattattcactaagttcaacaaatgttaattcttgttacagtcggttgcattccttggtcat

SEQ ID NO: 31 - DNA, 201 bp, Solanum lycopersicum
  source 1..201: mol_type = genomic DNA
agaaacaactaaattaagttgttgccatttgacaatataagccaacaataatttcgttgttgctaaaacgttgctgcgaattgtacattttcttgtagtgtgtgacagaaattgttgcttgtcttagcaaggtttacgatgatcatctcagcaggttagttttacatagcatccactaatttgytggaattttctgaaaaa

SEQ ID NO: 32 - DNA, 201 bp, Solanum lycopersicum
  source 1..201: mol_type = genomic DNA
ttttaaattggttccattttttactataaaattctttttgaatttgttttcgtgccagggatcctggactaaaatcaatgagtcgattaaacataattaagcatcattgagatcagttgatttatcaacactgaagtccatttctgactgagttggatccatatctgacaacttatcagttgcttgaacaatatttgttct

SEQ ID NO: 33 - DNA, 201 bp, Solanum lycopersicum
  source 1..201: mol_type = genomic DNA
gatggattcgtaaattcaatacgtgattccaagataagcatgttaattttaggaaaaaaatcttcaattttcttttaccatttttctttctttgggtggaaagattcctcgtcttcaaatggaaatactaaacgaaatgttactttgacaaaagaacgttccttctcttttggaggaatgacttcattatgatagtggact

SEQ ID NO: 34 - DNA, 201 bp, Solanum lycopersicum
  source 1..201: mol_type = genomic DNA
tgttactcttatatgaagttgtttacgttaatgaacatgttattggtcttacttctttatgaggtgataagtacttatgttacaagttatatgaagcaaacctttacttatggtctcctatcttatttattttgttgtgtaacacctaaatatgaactatggtgaacttgagcttcgtaagtgtttctttaattatatgaa

SEQ ID NO: 35 - DNA, 201 bp, Solanum lycopersicum
  source 1..201: mol_type = genomic DNA
tggtaatggaaataatagttacaatcacggaaagtcacatatttactgtgagttctaccattacaaaggtcacactaaagagacttacaagctttatgaccatcctaagaagaaagatggagcatcgatctatccctcatgttaaggttgtttctattggggaatcaactcactaaggctagagttatgactaggtcctat

SEQ ID NO: 36 - DNA, 201 bp, Solanum lycopersicum
  source 1..201: mol_type = genomic DNA
tttgcacatggccaagatatactagaaacgcattatagttttgttaaatgttttatcctaagttttggctrtaaggtaaactattactcaagcatggagcctgtcttaataatatacatattaatgtatagcagttctaacataggtttcaggctgcccctttcttcaacaattaacggggacttacaataccacatgctc

SEQ ID NO: 37 - DNA, 201 bp, Solanum lycopersicum
  source 1..201: mol_type = genomic DNA
ttatccttcccttggattttgagaaagccgcaaattcttaatttctcccattcgagttgactcgtagaaaaggcgaaaaggtcccgaagtttaaagaatcaaagaagattgaagaaattgaatggtttgggcaaaaagtccaaaaattttattttggaaaaatgttgtattttatttgggcctaagcccttttgtattgtt

SEQ ID NO: 38 - DNA, 201 bp, Solanum lycopersicum
  source 1..201: mol_type = genomic DNA
ccagatcgtgcttagattgatttttgaactccatttcagcagattcagtggtgagtcctcatcctctaaggacgatattcatgagtttctttttagtgtttggttcttttgtttcagtttttgctagacttttttggggcttatgccaacatttctagtcagtttagaggctattttcagacatagttagtttcagcttag

SEQ ID NO: 39 - DNA, 201 bp, Solanum lycopersicum
  source 1..201: mol_type = genomic DNA
acaccgatgcaactttgctttcattttgatatatgtcacactagaaacagtgctacattttaaatatttaaatgtagtgggagtattatatctatgtaaatttttttatgctattttttgggtttcatggaagttttttttcgatactttggccaaggacagtcccgtttaactatataattttttaaattttctaggatt

SEQ ID NO: 40 - DNA, 201 bp, Solanum lycopersicum
  source 1..201: mol_type = genomic DNA
gtccctccaaggcttcgcttgcttaaataatagggaaatatacatctttttggctgatcgctaagtatacttggcgatgcttaggtgtttctcttcatatcttttcatcattttttcacgttttgcgcctaagtgtcactgccaacactaaaacttcaaatacttgaaacttaagagttttcatcagacattgagatagaa

SEQ ID NO: 41 - DNA, 201 bp, Solanum lycopersicum
  source 1..201: mol_type = genomic DNA
aacattaaaatatgtgtatacgatgaatatatgatgttttcatgaggtttccttgatgaattttactagttgattatgaaggtgatcattgtgatttaggccgttaaaggtgtgatttaggctattaattctattgtcttgttttagtgttctagattgatctttttaattcaattgtcttgaaattaattgatcgtagta

SEQ ID NO: 42 - DNA, 201 bp, Solanum lycopersicum
  source 1..201: mol_type = genomic DNA
gtgtccaaggcaaacctacaacaaaatccacattgatgtcttcccacatccaagtaggaacttggatttcttggagtaaaccacctgacttttggtgttcagcttttacttcttggcaatttggagattttgcaacaaattccactatatccttcttcaagccttcccaccaaaacacttcgctaaggtcatggttcatct

SEQ ID NO: 43 - DNA, 201 bp, Solanum lycopersicum
  source 1..201: mol_type = genomic DNA
tctcctatggcctatacagatatatgatggttaatgaaggcttaaagacattttaaaaagggactttatcttagcaccgagcgaactaaatatgagaggtgttttttcccaatgtgggaaggtaggtttgtaatggttcttatgagatggagataacagtgcaatgttcataaagacggtctctagcatatatcctagtta

SEQ ID NO: 44 - DNA, 201 bp, Solanum lycopersicum
  source 1..201: mol_type = genomic DNA
tccatctttgaacatagtagtattttttctttagacttcatgttgttgggatatgtatgaaataatgttgttcacattcccaatatttcccgcatcaaccgaaaaattgttaatttttacgagctcttctcacctagatttctctatattaatcgattggatgaatttgctgatattagagtaaaccgataacctacatcc

SEQ ID NO: 45 - DNA, 201 bp, Solanum lycopersicum
  source 1..201: mol_type = genomic DNA
gtttgattagttgtttgtttataattttcgttttgggttcttcaagtgtgaagaactttagtttacctactgttattgtacgttatttggcagagaaaaacgtgagtgagagtaatagagacgtgagagagagagatgagcatgggagagaagagttttcttaggcttaggagtctagtttaggacttagtcaaataagtt

SEQ ID NO: 46 - DNA, 201 bp, Solanum lycopersicum
  source 1..201: mol_type = genomic DNA
atctgcaaacaaaaagtgacaacattaataggaggatmcattagccaagtkttgtgtgctttggaaaatcgacattgactaatggtacagaacatcaaccawcctaaacacatgtaacatgccatgtgcgcatcttgaaaacaactttgaccaatggaacgcaacatwagaaaaggccggtccactttgtgcaagaggcat

SEQ ID NO: 47 - DNA, 201 bp, Solanum lycopersicum
  source 1..201: mol_type = genomic DNA
gtttaggttagcgtgtagtggtattttttagggtgtggggttaaggatttgaagttaaatatctatggtgtagtgtttaattttttggattttgtatttttgtcatgaggtttagggtatagggtataggttaaagtgttatgattagggttagggctaaggttagaggtagggttawgatttagtgttcgagtttaggat

SEQ ID NO: 48 - DNA, 201 bp, Solanum lycopersicum
  source 1..201: mol_type = genomic DNA
aatgttgtcatgtttgctttaaaaatttatatataaaaatataaaagtattttatacaaaatatatagaaaaaattgaggagaaaaaaacttgatttttttaaaaaaattggaccaattggtgaaaaaaaattggctctaaaaactaaactctaaaatttaaatagtcatccaaatatatttatatttttaaaatctaaca

SEQ ID NO: 49 - DNA, 201 bp, Solanum lycopersicum
  source 1..201: mol_type = genomic DNA
tagaagatgatggactttctgatgtatctgagctgctattctcactttgtctatctttatttgaccatagttttgggaacatctttttggaccaattattaaagattgataaacttggatagtggtagatttggatctctagcaacttcagtatcgattaccttagccacctttactccggaatcatctgatgcaaacggg

SEQ ID NO: 50 - DNA, 201 bp, Solanum lycopersicum
  source 1..201: mol_type = genomic DNA
atatcataacatttaagagtacataacatcatgatactttaacaatatagaccaacacatattcataagtgacacaatcaacatatagtatcaacaatgttcaagtttatcatatgcatgccagataacattacaatcatattcatacataagaacatcctcctaagactcccttcaaggctaactagtgcgatgttttgt

SEQ ID NO: 51 - DNA, 201 bp, Solanum lycopersicum
  source 1..201: mol_type = genomic DNA
ctctcactttgaatattcagtttcctcatttcatcaataggaagtgttccttcccctatatttccctgataattgctcaaattagctccaaacacaccaccatttctactagctccaaaaacaaacccttcattaccaacatccccactacccctatcaaccccagaagcaaaacccacattcccaaatttcccaggaacc

SEQ ID NO: 52 - DNA, 111 bp, Solanum lycopersicum
  source 1..111: mol_type = genomic DNA
ggtattcactatcctgtattaatatctgttgcacatgttccagaacttaactatataagagttgaggatgatggcttagaaataggtgctggagttaagttgtcacagctt

SEQ ID NO: 53 - DNA, 201 bp, Solanum lycopersicum
  source 1..201: mol_type = genomic DNA
taaagtagcgtgtaaccattggtgatgcatgtaaagggaattttctaaatacaatcattttttcttcaaagttaaccatttgtagctttaactgttcaatagccttgcacataaggtgtatccttcttggccctctgtttagacaaagtaccatcaataggatgagagttacagaaaaaagtagcagaagtacttctcaga